European Patent Application EP 4 349 374 A1, published April 10, 2024. Title: Anti-urokinase plasminogen activator receptor immunoglobulin single variable domains. Applicant: Vrije Universiteit Brussel. The sequence listing filed with the application follows.

SEQUENCE LISTING (23 sequences)

SEQ ID NO: 1 - protein, 335 aa, Homo sapiens
MGHPPLLPLLLLLHTCVPASWGLRCMQCKTNGDCRVEECALGQDLCRTTIVRLWEEGEELELVEKSCTHSEKTNRTLSYRTGLKITSLTEVVCGLDLCNQGNSGRAVTYSRSRYLECISCGSSDMSCERGRHQSLQCRSPEEQCLDVVTHWIQEGEEGRPKDDRHLRGCGYLPGCPGSNGFHNNDTFHFLKCCNTTKCNEGPILELENLPQNGRQCYSCKGNSTHGCSSEETFLIDCRGPMNQCLVATGTHEPKNQSYMVRGCATASMCQHAHLGDAFSMNHIDVSCCTKSGCNHPDLDVQYRSGAAPQPGPAHLSLTITLLMTARLWGGTLLWT

SEQ ID NO: 2 - protein, 126 aa, Vicugna pacos
QVQLQESGGGWVQPGGSLRLSCAASGFTLDYYGIGWFRQAPGKEREGVSCISSSDGSTYYADSVKGRFTISRDNAKNTVYLQMNSLKPEDTAVYYCATRGASCYYTGSYSLGYDYWGQGTQVTVSS

SEQ ID NO: 3 - protein, 8 aa, Vicugna pacos
GFTLDYYG

SEQ ID NO: 4 - protein, 8 aa, Vicugna pacos
ISSSDGST

SEQ ID NO: 5 - protein, 19 aa, Vicugna pacos
ATRGASCYYTGSYSLGYDY

SEQ ID NO: 6 - protein, 25 aa, Vicugna pacos
QVQLQESGGGWVQPGGSLRLSCAAS

SEQ ID NO: 7 - protein, 17 aa, Vicugna pacos
IGWFRQAPGKEREGVSC

SEQ ID NO: 8 - protein, 38 aa, Vicugna pacos
YYADSVKGRFTISRDNAKNTVYLQMNSLKPEDTAVYYC

SEQ ID NO: 9 - protein, 11 aa, Vicugna pacos
WGQGTQVTVSS

SEQ ID NO: 10 - protein, 335 aa, Canis lupus
MGHPLLLPLLGLLLQTCVPVSWSLQCMLCGSTGKCQVEECTPGQDLCRTTIMRIWEDGDELEVVERGCTHPEKSNRTMSYRTGMKIITLTEAVCGTNLCNKPTSGRVSTFPRTRSRYLECVSCGSSDLSCERGLDQSLQCRSPTEQCVEVVTHRGLEDSPKDEHHTRGCGNLPGCPGPTGFHNNHTFHFLQCCNTTKCNAGPVLELQNLPLNGLQCFGCEGNSTHGCSSEETSLIACRGPMNQCLDATGTNGLGNPSYTVRGCATPSWCQSLHVAEAFSMTHLNVSCCTGNSCNHPILDHQPRIGSAPRPGPAHLSLTVTLLLTARLWGGTLLWT

SEQ ID NO: 11 - protein, 10 aa, synthetic construct
GSGSGSGSGS

SEQ ID NO: 12 - protein, 20 aa, synthetic construct
GSGSGSGSGSGSGSGSGSGS

SEQ ID NO: 13 - protein, 15 aa, synthetic construct
GGGGSGGGGSGGGGS

SEQ ID NO: 14 - protein, 17 aa, synthetic construct
AHHSEDPSSKAPKAPMA

SEQ ID NO: 15 - protein, 16 aa, synthetic construct
SPSTPPTPSPSTPPAS

SEQ ID NO: 16 - protein, 4 aa, synthetic construct
IEGR

SEQ ID NO: 17 - protein, 4 aa, synthetic construct
LVPR

SEQ ID NO: 18 - protein, 5 aa, synthetic construct
DDDDK

SEQ ID NO: 19 - protein, 8 aa, synthetic construct
LEVLFQGP

SEQ ID NO: 20 - protein, 126 aa, Vicugna pacos
QVQLQESGGGLVQPGGSLRLSCAISGFTLDYYGIGWFRQAPGKEREGVSCISSSDGSTYYADSVKGRFTISRDNAKNTVYLQMNSLKPEDTAVYYCATRGASCYYSGSYSLGYDYWGQGTQVTVSS

SEQ ID NO: 21 - protein, 126 aa, Vicugna pacos
QVQLQESGGGLVQPGGSLRLSCAVSGSTLEYYGIGWFRQAPGKEREGVSCISSSDGSTYYADSVKGRFTISRDNAKNTVYLQMNSLKPEDTAVYYCATRGASCYYTGSYSLGYDYWGQGTQVTVSS

SEQ ID NO: 22 - protein, 126 aa, Vicugna pacos
QVQLQESGGGLAQPGGSLRLSCTASGFTSDYYGIGWFRQAPGKEREGVSCISSSDGSTYYADSVKGRFTISRDNAKNTVYLQMNSLKPEDTAVYYCATRGASCYYTGSYSLGYDYWGQGTQVTVSS

SEQ ID NO: 23 - protein, 283 aa, Vicugna pacos
LRCMQCKTNGDCRVEECALGQDLCRTTIVRLWEEGEELELVEKSCTHSEKTNRTLSYRTGLKITSLTEVVCGLDLCNQGNSGRAVTYSRSRYLECISCGSSDMSCERGRHQSLQCRSPEEQCLDVVTHWIQEGEEGRPKDDRHLRGCGYLPGCPGSNGFHNNDTFHFLKCCNTTKCNEGPILELENLPQNGRQCYSCKGNSTHGCSSEETFLIDCRGPMNQCLVATGTHEPKNQSYMVRGCATASMCQHAHLGDAFSMNHIDVSCCTKSGCNHPDLDVQYRSG